European Patent Application EP 4 205 757 A1, published July 5, 2023. Title: Expression vector for cholesterol 24-hydrolase in therapy of amyotrophic lateral sclerosis. Applicant: INSERM. Application EP. The sequence listing filed with the application follows.

SEQUENCE LISTING (23 sequences)

SEQ ID NO: 1 - DNA, 1503 bp, Homo sapiens
  source 1..1503: mol_type = genomic DNA
atgagccccgggctgctgctgctcggtagcgccgtcctgctcgccttcggcctctgctgcaccttcgtgcaccgcgctcgcagccgctacgagcacatccccgggccgccgcggcccagtttccttctaggacacctcccctgcttttggaaaaaggatgaggttggtggccgtgtgctccaagatgtgtttttggattgggctaagaagtatggacctgttgtgcgggtcaacgtcttccacaaaacctcagtcatcgtcacgagtcctgagtcggttaagaagttcctgatgtcaaccaagtacaacaaggactccaagatgtaccgtgcgctccagactgtgtttggtgagagactcttcggccaaggcttggtgtccgaatgcaactatgagcgctggcacaagcagcggagagtcatagacctggccttcagccggagctccttggttagcttaatggaaacattcaacgagaaggctgagcagctggtggagattctagaagccaaggcagatgggcagaccccagtgtccatgcaggacatgctgacctacaccgccatggacatcctggccaaggcagcttttgggatggagaccagtatgctgctgggtgcccagaagcctctgtcccaggcagtgaaacttatgttggagggaatcactgcgtcccgcaacactctggcaaagttcctgccagggaagaggaagcagctccgggaggtccgggagagcattcgcttcctgcgccaggtgggcagggactgggtccagcgccgccgggaagccctgaagaggggcgaggaggttcctgccgacatcctcacacagattctgaaagctgaagagggagcccaggacgacgagggtctgctggacaacttcgtcaccttcttcattgctggtcacgagacctctgccaaccacttggcgttcacagtgatggagctgtctcgccagccagagatcgtggcaaggctgcaggccgaggtggatgaggtcattggttctaagaggtacctggatttcgaggacctggggagactgcagtacctgtcccaggtcctcaaagagtcgctgaggctgtacccaccagcatggggcacctttcgcctgctggaagaggagaccttgattgatggggtcagagtccccggcaacaccccgctcttgttcagcacctatgtcatggggcggatggacacatactttgaggacccgctgactttcaaccccgatcgcttcggccctggagcacccaagccacggttcacctacttccccttctccctgggccaccgctcctgcatcgggcagcagtttgctcagatggaggtgaaggtggtcatggcaaagctgctgcagaggctggagttccggctggtgcccgggcagcgcttcgggctgcaggagcaggccacactcaagccactggaccccgtgctgtgcaccctgcggccccgcggctggcagcccgcacccccaccacccccctgctga

SEQ ID NO: 2 - protein, 500 aa, Homo sapiens
MSPGLLLLGSAVLLAFGLCCTFVHRARSRYEHIPGPPRPSFLLGHLPCFWKKDEVGGRVLQDVFLDWAKKYGPVVRVNVFHKTSVIVTSPESVKKFLMSTKYNKDSKMYRALQTVFGERLFGQGLVSECNYERWHKQRRVIDLAFSRSSLVSLMETFNEKAEQLVEILEAKADGQTPVSMQDMLTYTAMDILAKAAFGMETSMLLGAQKPLSQAVKLMLEGITASRNTLAKFLPGKRKQLREVRESIRFLRQVGRDWVQRRREALKRGEEVPADILTQILKAEEGAQDDEGLLDNFVTFFIAGHETSANHLAFTVMELSRQPEIVARLQAEVDEVIGSKRYLDFEDLGRLQYLSQVLKESLRLYPPAWGTFRLLEEETLIDGVRVPGNTPLLFSTYVMGRMDTYFEDPLTFNPDRFGPGAPKPRFTYFPFSLGHRSCIGQQFAQMEVKVVMAKLLQRLEFRLVPGQRFGLQEQATLKPLDPVLCTLRPRGWQPAPPPPPC

SEQ ID NO: 3 - DNA, 21 bp, synthetic construct
  misc_feature 1..21: note = primer
  source 1..21: mol_type = other DNA
tcctgagcgcaagtactctgt

SEQ ID NO: 4 - DNA, 21 bp, synthetic construct
  misc_feature 1..21: note = primer
  source 1..21: mol_type = other DNA
ctgatccacatctgctggaag

SEQ ID NO: 5 - DNA, 24 bp, synthetic construct
  misc_feature 1..24: note = primer
  source 1..24: mol_type = other DNA
agatcattgtcactcactttccct

SEQ ID NO: 6 - DNA, 23 bp, synthetic construct
  misc_feature 1..23: note = primer
  source 1..23: mol_type = other DNA
acgaagtggtaggtgatgtccag

SEQ ID NO: 7 - DNA, 22 bp, synthetic construct
  misc_feature 1..22: note = primer
  source 1..22: mol_type = other DNA
tcatcaccacgcctcttgaaac

SEQ ID NO: 8 - DNA, 23 bp, synthetic construct
  misc_feature 1..23: note = primer
  source 1..23: mol_type = other DNA
catcatcactgtcttccacgctc

SEQ ID NO: 9 - DNA, 28 bp, synthetic construct
  misc_feature 1..28: note = primer
  source 1..28: mol_type = other DNA
ggctaagaagtatggtcctgttgtaaga

SEQ ID NO: 10 - DNA, 25 bp, synthetic construct
  misc_feature 1..25: note = primer
  source 1..25: mol_type = other DNA
ggtggacatcaggaacttcttgact

SEQ ID NO: 11 - DNA, 24 bp, synthetic construct
  misc_feature 1..24: note = primer
  source 1..24: mol_type = other DNA
gtcacattgctgacaggatgccta

SEQ ID NO: 12 - DNA, 21 bp, synthetic construct
  misc_feature 1..21: note = primer
  source 1..21: mol_type = other DNA
gggttggttgctttgccactc

SEQ ID NO: 13 - DNA, 24 bp, synthetic construct
  misc_feature 1..24: note = primer
  source 1..24: mol_type = other DNA
ccccacattcactcttgacgctct

SEQ ID NO: 14 - DNA, 19 bp, synthetic construct
  misc_feature 1..19: note = primer
  source 1..19: mol_type = other DNA
gctggcggacgcctgacat

SEQ ID NO: 15 - DNA, 21 bp, synthetic construct
  misc_feature 1..21: note = primer
  source 1..21: mol_type = other DNA
ggtccagcaggtcccagttgt

SEQ ID NO: 16 - DNA, 21 bp, synthetic construct
  misc_feature 1..21: note = primer
  source 1..21: mol_type = other DNA
ctgcagtcttcacggtggctc

SEQ ID NO: 17 - DNA, 21 bp, synthetic construct
  misc_feature 1..21: note = primer
  source 1..21: mol_type = other DNA
tgttgacgcagacagccaatg

SEQ ID NO: 18 - DNA, 20 bp, synthetic construct
  misc_feature 1..20: note = primer
  source 1..20: mol_type = other DNA
cgctctctgctcctcctgtt

SEQ ID NO: 19 - DNA, 20 bp, synthetic construct
  misc_feature 1..20: note = primer
  source 1..20: mol_type = other DNA
ccatggtgtctgagcgatgt

SEQ ID NO: 20 - DNA, 25 bp, synthetic construct
  misc_feature 1..25: note = primer
  source 1..25: mol_type = other DNA
cgagtcctgagtcggttaagaagtt

SEQ ID NO: 21 - DNA, 21 bp, synthetic construct
  misc_feature 1..21: note = primer
  source 1..21: mol_type = other DNA
agtctggagcgcacggtacat

SEQ ID NO: 22 - DNA, 20 bp, synthetic construct
  misc_feature 1..20: note = primer
  source 1..20: mol_type = other DNA
ccacctctcctatgggcaga

SEQ ID NO: 23 - DNA, 19 bp, synthetic construct
  misc_feature 1..19: note = primer
  source 1..19: mol_type = other DNA
ccgggccttttcaatgtct